European Patent Specification EP 3 929 305 B1, published November 8, 2023. Title: MULTIPLEX RNA REFERENCE MATERIALS. Applicant: SERACARE LIFE SCIENCES, INC. The sequence listing filed with the application follows.

SEQUENCE LISTING (13 sequences)

SEQ ID NO: 1 - DNA, 3900 bp, Homo sapiens
ggcggcgcggcgcggcgctcgcggctgctgcctgggagggaggccgggcaggcggctgagcggcgcggctctcaacgtgacggggaagtggttcgggcggccgcggcttactaccccagggcgaacggacggacgacggaggcgggagccggtagccgagccgggcgacctagagaacgagcgggtcaggctcagcgtcggccactctgtcggtccgctgaatgaagtgcccgcccctctgagcccggagcccggcgctttccccgcaagatggacggtttcgccggcagtctcgatgatagtatttctgctgcaagtacttctgatgttcaagatcgcctgtcagctcttgagtcacgagttcagcaacaagaagatgaaatcactgtgctaaaggcggctttggctgatgttttgaggcgtcttgcaatctctgaagatcatgtggcctcagtgaaaaaatcagtctcaagtaaaggccaaccaagccctcgagcagttattcccatgtcctgtataaccaatggaagtggtgcaaacagaaaaccaagtcataccagtgctgtctcaattgcaggaaaagaaactctttcatctgctgctaaaagtggtacagaaaaaaagaaagaaaaaccacaaggacagagagaaaaaaaagaggaatctcattctaatgatcaaagtccacaaattcgagcatcaccttctccccagccctcttcacaacctctccaaatacacagacaaactccagaaagcaagaatgctactcccaccaaaagcataaaacgaccatcaccagctgaaaagtcacataattcttgggaaaattcagatgatagccgtaataaattgtcgaaaataccttcaacacccaaattaataccaaaagttaccaaaactgcagacaagcataaagatgtcatcatcaaccaagaaggagaatatattaaaatgtttatgcgcggtcggccaattaccatgttcattccttccgatgttgacaactatgatgacatcagaacggaactgcctcctgagaagctcaaactggagtgggcatatggttatcgaggaaaggactgtagagctaatgtttaccttcttccgaccggggaaatagtttatttcattgcatcagtagtagtactatttaattatgaggagagaactcagcgacactacctgggccatacagactgtgtgaaatgccttgctatacatcctgacaaaattaggattgcaactggacagatagctggcgtggataaagatggaaggcctctacaaccccacgtcagagtgtgggattctgttactctatccacactgcagattattggacttggcacttttgagcgtggagtaggatgcctggatttttcaaaagcagattcaggtgttcatttatgtgttattgatgactccaatgagcatatgcttactgtatgggactggcagaagaaagcaaaaggagcagaaataaagacaacaaatgaagttgttttggctgtggagtttcacccaacagatgcaaataccataattacatgcggtaaatctcatattttcttctggacctggagcggcaattcactaacaagaaaacagggaatttttgggaaatatgaaaagccaaaatttgtgcagtgtttagcattcttggggaatggagatgttcttactggagactcaggtggagtcatgcttatatggagcaaaactactgtagagcccacacctgggaaaggacctaaagtgtaccgccggaagcaccaggagctgcaagccatgcagatggagctgcagagccctgagtacaagctgagcaagctccgcacctcgaccatcatgaccgactacaaccccaactactgctttgctggcaagacctcctccatcagtgacctgaaggaggtgccgcggaaaaacatcaccctcattcggggtctgggccatggagcctttggggaggtgtatgaaggccaggtgtccggaatgcccaacgacccaagccccctgcaagtggctgtgaagacgctgcctgaagtgtgctctgaacaggacgaactggatttcctcatggaagccctgatcatcagcaaattcaaccaccagaacattgttcgctgcattggggtgagcctgcaatccctgccccggttcatcctgctggagctcatggcggggggagacctcaagtccttcctccgagagacccgccctcgcccgagccagccctcctccctggccatgctggaccttctgcacgtggctcgggacattgcctgtggctgtcagtatttggaggaaaaccacttcatccaccgagacattgctgccagaaactgcctcttgacctgtccaggccctggaagagtggccaagattggagacttcgggatggcccgagacatctacagggcgagctactatagaaagggaggctgtgccatgctgccagttaagtggatgcccccagaggccttcatggaaggaatattcacttctaaaacagacacatggtcctttggagtgctgctatgggaaatcttttctcttggatatatgccataccccagcaaaagcaaccaggaagttctggagtttgtcaccagtggaggccggatggacccacccaagaactgccctgggcctgtataccggataatgactcagtgctggcaacatcagcctgaagacaggcccaactttgccatcattttggagaggattgaatactgcacccaggacccggatgtaatcaacaccgctttgccgatagaatatggtccacttgtggaagaggaagagaaagtgcctgtgaggcccaaggaccctgagggggttcctcctctcctggtctctcaacaggcaaaacgggaggaggagcgcagcccagctgccccaccacctctgcctaccacctcctctggcaaggctgcaaagaaacccacagctgcagaggtctctgttcgagtccctagagggccggccgtggaagggggacacgtgaatatggcattctctcagtccaaccctccttcggagttgcacagggtccacggatccagaaacaagcccaccagcttgtggaacccaacgtacggctcctggtttacagagaaacccaccaaaaagaataatcctatagcaaagaaggagccacacgagaggggtaacctggggctggagggaagctgtactgtcccacctaacgttgcaactgggagacttccgggggcctcactgctcctagagccctcttcgctgactgccaatatgaaggaggtacctctgttcaggctacgtcacttcccttgtgggaatgtcaattacggctaccagcaacagggcttgcccttagaagccgctactgcccctggagctggtcattacgaggataccattctgaaaagcaagaatagcatgaaccagcctgggccctgagctcggtcacacactcacttctcttccttgggatccctaagaccgtggaggagagagaggcaatcaatggctccttcacaaaccagagaccaaatgtcacgttttgttttgtgccaacctattttgaagtaccaccaaaaaagctgtattttgaaaatgctttagaaaggttttgagcatgggttcatcctattctttcgaaagaagaaaatatcataaaaatgagtgataaatacaaggcccagatgtggttgcataaggtttttatgcatgtttgttgtatacttccttatgcttcttttaaattgtgtgtgctctgcttcaatgtagtcagaattagctgcttctatgtttcatagttggggtcatagatgtttccttgccttgttgatgtggacatgagccatttgaggggagagggaacggaaataaaggagttatttgtaatga

SEQ ID NO: 2 - DNA, 2043 bp, Homo sapiens
atggaagattcgatggacatggacatgagccccctgaggccccagaactatcttttcggttgtgaactaaaggccgacaaagattatcactttaaggtggataatgatgaaaatgagcaccagttatctttaagaacggtcagtttaggggctggtgcaaaggatgagttgcacattgttgaagcagaggcaatgaattacgaaggcagtccaattaaagtaacactggcaactttgaaaatgtctgtacagccaacggtttcccttgggggctttgaaataacaccaccagtggtcttaaggttgaagtgtggttcagggccagtgcatattagtggacagcacttagtagtgtaccgccggaagcaccaggagctgcaagccatgcagatggagctgcagagccctgagtacaagctgagcaagctccgcacctcgaccatcatgaccgactacaaccccaactactgctttgctggcaagacctcctccatcagtgacctgaaggaggtgccgcggaaaaacatcaccctcattcggggtctgggccatggcgcctttggggaggtgtatgaaggccaggtgtccggaatgcccaacgacccaagccccctgcaagtggctgtgaagacgctgcctgaagtgtgctctgaacaggacgaactggatttcctcatggaagccctgatcatcagcaaattcaaccaccagaacattgttcgctgcattggggtgagcctgcaatccctgccccggttcatcctgctggagctcatggcggggggagacctcaagtccttcctccgagagacccgccctcgcccgagccagccctcctccctggccatgctggaccttctgcacgtggctcgggacattgcctgtggctgtcagtatttggaggaaaaccacttcatccaccgagacattgctgccagaaactgcctcttgacctgtccaggccctggaagagtggccaagattggagacttcgggatggcccgagacatctacagggcgagctactatagaaagggaggctgtgccatgctgccagttaagtggatgcccccagaggccttcatggaaggaatattcacttctaaaacagacacatggtcctttggagtgctgctatgggaaatcttttctcttggatatatgccataccccagcaaaagcaaccaggaagttctggagtttgtcaccagtggaggccggatggacccacccaagaactgccctgggcctgtataccggataatgactcagtgctggcaacatcagcctgaagacaggcccaactttgccatcattttggagaggattgaatactgcacccaggacccggatgtaatcaacaccgctttgccgatagaatatggtccacttgtggaagaggaagagaaagtgcctgtgaggcccaaggaccctgagggggttcctcctctcctggtctctcaacaggcaaaacgggaggaggagcgcagcccagctgccccaccacctctgcctaccacctcctctggcaaggctgcaaagaaacccacagctgcagaggtctctgttcgagtccctagagggccggccgtggaagggggacacgtgaatatggcattctctcagtccaaccctccttcggagttgcacaaggtccacggatccagaaacaagcccaccagcttgtggaacccaacgtacggctcctggtttacagagaaacccaccaaaaagaataatcctatagcaaagaaggagccacacgacaggggtaacctggggctggagggaagctgtactgtcccacctaacgttgcaactgggagacttccgggggcctcactgctcctagagccctcttcgctgactgccaatatgaaggaggtacctctgttcaggctacgtcacttcccttgtgggaatgtcaattacggctaccagcaacagggcttgcccttagaagccgctactgcccctggagctggtcattacgaggataccattctgaaaagcaagaatagcatgaaccagcctgggccctga

SEQ ID NO: 3 - DNA, 4400 bp, Homo sapiens
cggaagtgagcattagggttaacggctgccggcgccggctcttcaagtcccggctccccggccgcctccacccggggaagcgcagcgcggcgcagctgactgctgcctctcacggccctcgcgaccacaagccctcaggtccggcgcgttccctgcaagactgagcggcggggagtggctcccggccgccggccccggctgcgagaaagatggcggacctggccgagtgcaacatcaaagtgatgtgtcgcttcagacctctcaacgagtctgaagtgaaccgcggcgacaagtacatcgccaagtttcagggagaagacacggtcgtgatcgcgtccaagccttatgcatttgatcgggtgttccagtcaagcacatctcaagagcaagtgtataatgactgtgcaaagaagattgttaaagatgtacttgaaggatataatggaacaatatttgcatatggacaaacatcctctgggaagacacacacaatggagggtaaacttcatgatccagaaggcatgggaattattccaagaatagtgcaagatatttttaattatatttactccatggatgaaaatttggaatttcatattaaggtttcatattttgaaatatatttggataagataagggacctgttagatgtttcaaagaccaacctttcagttcatgaagacaaaaaccgagttccctatgtaaaggggtgcacagagcgttttgtatgtagtccagatgaagttatggataccatagatgaaggaaaatccaacagacatgtagcagttacaaatatgaatgaacatagctctaggagtcacagtatatttcttattaatgtcaaacaagagaacacacaaacggaacaaaagctgagtggaaaactttatctggttgatttagctggtagtgaaaaggttagtaaaactggagctgaaggtgctgtgctggatgaagctaaaaacatcaacaagtcactttctgctcttggaaatgttatttctgctttggctgagggtagtacatatgttccatatcgagatagtaaaatgacaagaatccttcaagattcattaggtggcaactgtagaaccactattgtaatttgctgctctccatcatcatacaatgagtctgaaacaaaatctacactcttatttggccaaagggccaaaacaattaagaacacagtttgtgtcaatgtggagttaactgcagaacagtggaaaaagaagtatgaaaaagaaaaagaaaaaaataagatcctgcggaacactattcagtggcttgaaaatgagctcaacagatggcgtaatggggagacggtgcctattgatgaacagtttgacaaagagaaagccaacttggaagctttcacagtggataaagatattactcttaccaatgataaaccagcaaccgcaattggagttataggaaattttactgatgctgaaagaagaaagtgtgaagaagaaattgctaaattatacaaacagcttgatgacaaggatgaagaaattaaccagcaaagtcaactggtagagaaactgaagacgcaaatgttggatcaggaggagcttttggcatctaccagaagggatcaagacaatatgcaagctgagctgaatcgccttcaagcagaaaatgatgcctctaaagaagaagtgaaagaagttttacaggccctagaagaacttgctgtcaattatgatcagaagtctcaggaagttgaagacaaaactaaggaatatgaattgcttagtgatgaattgaatcagaaatcggcaactttagcgagtatagatgctgagcttcagaaacttaaggaaatgaccaaccaccagaaaaaacgagcagctgagatgatggcatctttactaaaagaccttgcagaaataggaattgctgtgggaaataatgatgtaaagcagcctgagggaactggcatgatagatgaagagttcactgttgcaagactctacattagcaaaatgaagtcagaagtaaaaaccatggtgaaacgttgcaagcagttagaaagcacacaaactgagagcaacaaaaaaatggaagaaaatgaaaaggagttagcagcatgtcagcttcgtatctctcaacatgaagccaaaatcaagtcattgactgaataccttcaaaatgtggaacaaaagaaaagacagttggaggaatctgtcgatgccctcagtgaagaactagtccagcttcgagcacaagagaaagtccatgaaatggaaaaggagcacttaaataaggttcagactgcaaatgaagttaagcaagctgttgaacagcagatccagagccatagagaaactcatcaaaaacagatcagtagtttgagagatgaagtagaagcaaaagcaaaacttattactgatcttcaagaccaaaaccagaaaatgatgttagagcaggaacgtctaagagtagaacatgagaagttgaaagccacagatcaggaaaagagcagaaaactacatgaacttacggttatgcaagatagacgagaacaagcaagacaagacttgaagggtttggaagagacagtggcaaaagaacttcagactttacacaacctgcgcaaactctttgttcaggacctggctacaagagttaaaaagagtgctgagattgattctgatgacaccggaggcagcgctgctcagaagcaaaaaatctcctttcttgaaaataatcttgaacagctcactaaagtgcacaaacagttggtacgtgataatgcagatctccgctgtgaacttcctaagttggaaaagcgacttcgagctacagctgagagagtgaaagctttggaatcagcactgaaagaagctaaagaaaatgcatctcgtgatcgcaaacgctatcagcaagaagtagatcgcataaaggaagcagtcaggtcaaagaatatggccagaagagggcattctgcacagattgatccactgtgcgacgagctgtgccgcacggtgatcgcagccgctgtcctcttctccttcatcgtctcggtgctgctgtctgccttctgcatccactgctaccacaagtttgcccacaagccacccatctcctcagctgagatgaccttccggaggcccgcccaggccttcccggtcagctactcctcttccggtgcccgccggccctcgctggactccatggagaaccaggtctccgtggatgccttcaagatcctggaggatccaaagtgggaattccctcggaagaacttggttcttggaaaaactctaggagaaggcgaatttggaaaagtggtcaaggcaacggccttccatctgaaaggcagagcagggtacaccacggtggccgtgaagatgctgaaagagaacgcctccccgagtgagcttcgagacctgctgtcagagttcaacgtcctgaagcaggtcaaccacccacatgtcatcaaattgtatggggcctgcagccaggatggcccgctcctcctcatcgtggagtacgccaaatacggctccctgcggggcttcctccgcgagagccgcaaagtggggcctggctacctgggcagtggaggcagccgcaactccagctccctggaccacccggatgagcgggccctcaccatgggcgacctcatctcatttgcctggcagatctcacaggggatgcagtatctggccgagatgaagctcgttcatcgggacttggcagccagaaacatcctggtagctgaggggcggaagatgaagatttcggatttcggcttgtcccgagatgtttatgaagaggattcctacgtgaagaggagccagggtcggattccagttaaatggatggcaattgaatccctttttgatcatatctacaccacgcaaagtgatgtatggtcttttggtgtcctgctgtgggagatcgtgaccctagggggaaacccctatcctgggattcctcctgagcggctcttcaaccttctgaagaccggccaccggatggagaggccagacaactgcagcgaggagatgtaccgcctgatgctgcaatgctggaagcaggagccggacaaaaggccggtgtttgcggacatcagcaaagacctggagaagatgatggttaagaggagagactacttggaccttgcggcgtccactccatctgactccctgatttatgacgacggcctctcagaggaggagacaccgctggtggactgtaataatgcccccctccctcgagccctcccttccacatggattgaaaacaaactctatggtagaatttcccatgcatttactagattctagcaccgctgtcccctctgcactatccttcctctctgtgatgctttttaaaaatgtttctggtctgaacaaaaccaaagtctgctctgaacc

SEQ ID NO: 4 - DNA, 900 bp, Homo sapiens
tctcagtccacccaaggtctcctcggatcgcctggagaggcactcggacctggagcagtgaggagaatgaataccttccaagaccagagtggcagctccagtaatagagaaccccttttgaggtgtagtgatgcacggagggacttggagcttgctattggtggagttctccgggctgaacagcaaattaaagataacttgcgagaggtcaaagctcagattcacagttgcataagccgtcacctggaatgtcttagaagccgtgaggtatggctgtatgaacaggtggaccttatttatcagcttaaagaggagacacttcaacagcaggctcagcagctctactcgttattgggccagttcaattgtcttactcatcaactggagtgtacccaaaacaaagatctagccaatcaagtctctgtgtgcctggagagactgggcagtttgacccttaagcctgaagattcaactgtcctgctctttgaagctgacacaattactctgcgccagaccatcaccacatttgggtctctcaaaaccattcaaattcctgagcacttgatggctcatgctagttcagcaaatattgggcccttcctggagaagagaggctgtatctccatgccagagcagaagtcagcatccggtattgtagctgtccctttcagcgaatggctccttggaagcaaacctgccagtggttatcaagctccttacatacccagcaccgacccccaggactggcttatccaaaagcagaccttggagaacagtcaggaggatccaaagtgggaattccctcggaagaacttggttcttggaaaaactctaggagaaggcgaatttggaaaagtggtcaaggcaacggccttccatctgaaaggcagagcagggtac

SEQ ID NO: 5 - DNA, 2112 bp, Homo sapiens
atgcacaggaggagaagcaggagctgtcgggaagatcagaagccagtcatggatgaccagcgcgaccttatctccaacaatgagcaactgcccatgctgggccggcgccctggggccccggagagcaagtgcagccgcggagccctgtacacaggcttttccatcctggtgactctgctcctcgctggccaggccaccaccgcctacttcctgtaccagcagcagggccggctggacaaactgacagtcacctcccagaacctgcagctggagaacctgcgcatgaagcttcccaagcctcccaagcctgtgagcaagatgcgcatggccaccccgctgctgatgcaggcgctgcccatgggagccctgccccaggggcccatgcagaatgccaccaagtatggcaacatgacagaggaccatgtgatgcacctgctccagaatgctgaccccctgaaggtgtacccgccactgaaggggagcttcccggagaacctgagacaccttaagaacaccatggagaccatagactggaaggtctttgagagctggatgcaccattggctcctgtttgaaatgagcaggcactccttggagcaaaagcccactgacgctccaccgaaagatgatttttggataccagaaacaagtttcatacttactattatagttggaatatttctggttgttacaatcccactgacctttgtctggcatagaagattaaagaatcaaaaaagtgccaaggaaggggtgacagtgcttataaacgaagacaaagagttggctgagctgcgaggtctggcagccggagtaggcctggctaatgcctgctatgcaatacatactcttccaacccaagaggagattgaaaatcttcctgccttccctcgggaaaaactgactctgcgtctcttgctgggaagtggagcctttggagaagtgtatgaaggaacagcagtggacatcttaggagttggaagtggagaaatcaaagtagcagtgaagactttgaagaagggttccacagaccaggagaagattgaattcctgaaggaggcacatctgatgagcaaatttaatcatcccaacattctgaagcagcttggagtttgtctgctgaatgaaccccaatacattatcctggaactgatggagggaggagaccttcttacttatttgcgtaaagcccggatggcaacgttttatggtcctttactcaccttggttgaccttgtagacctgtgtgtagatatttcaaaaggctgtgtctacttggaacggatgcatttcattcacagggatctggcagctagaaattgccttgtttccgtgaaagactataccagtccacggatagtgaagattggagactttggactcgccagagacatctataaaaatgattactatagaaagagaggggaaggcctgctcccagttcggtggatggctccagaaagtttgatggatggaatcttcactactcaatctgatgtatggtcttttggaattctgatttgggagattttaactcttggtcatcagccttatccagctcattccaaccttgatgtgttaaactatgtgcaaacaggagggagactggagccaccaagaaattgtcctgatgatctgtggaatttaatgacccagtgctgggctcaagaacccgaccaaagacctacttttcatagaattcaggaccaacttcagttattcagaaattttttcttaaatagcatttataagtccagagatgaagcaaacaacagtggagtcataaatgaaagctttgaaggtgaagatggcgatgtgatttgtttgaattcagatgacattatgccagttgctttaatggaaacgaagaaccgagaagggttaaactatatggtacttgctacagaatgtggccaaggtgaagaaaagtctgagggtcctctaggctcccaggaatctgaatcttgtggtctgaggaaagaagagaaggaaccacatgcagacaaagatttctgccaagaaaaacaagtggcttactgcccttctggcaagcctgaaggcctgaactatgcctgtctcactcacagtggatatggagatgggtctgattaa

SEQ ID NO: 6 - DNA, 1866 bp, Homo sapiens
atggctccctggcctgaattgggagatgcccagcccaaccccgataagtacctcgaaggggccgcaggtcagcagcccactgcccctgataaaagcaaagagaccaacaaaacagataacactgaggcacctgtaaccaagattgaacttctgccgtcctactccacggctacactgatagatgagcccactgaggtggatgacccctggaacctacccactcttcaggactcggggatcaagtggtcagagagagacaccaaagggaagattctctgtttcttccaagggattgggagattgattttacttctcggatttctctactttttcgtgtgctccctggatattcttagtagcgccttccagctggttggagatgatttttggataccagaaacaagtttcatacttactattatagttggaatatttctggttgttacaatcccactgacctttgtctggcatagaagattaaagaatcaaaaaagtgccaaggaaggggtgacagtgcttataaacgaagacaaagagttggctgagctgcgaggtctggcagccggagtaggcctggctaatgcctgctatgcaatacatactcttccaacccaagaggagattgaaaatcttcctgccttccctcgggaaaaactgactctgcgtctcttgctgggaagtggagcctttggagaagtgtatgaaggaacagcagtggacatcttaggagttggaagtggagaaatcaaagtagcagtgaagactttgaagaagggttccacagaccaggagaagattgaattcctgaaggaggcacatctgatgagcaaatttaatcatcccaacattctgaagcagcttggagtttgtctgctgaatgaaccccaatacattatcctggaactgatggagggaggagaccttcttacttatttgcgtaaagcccggatggcaacgttttatggtcctttactcaccttggttgaccttgtagacctgtgtgtagatatttcaaaaggctgtgtctacttggaacggatgcatttcattcacagggatctggcagctagaaattgccttgtttccgtgaaagactataccagtccacggatagtgaagattggagactttggactcgccagagacatctataaaaatgattactatagaaagagaggggaaggcctgctcccagttcggtggatggctccagaaagtttgatggatggaatcttcactactcaatctgatgtatggtcttttggaattctgatttgggagattttaactcttggtcatcagccttatccagctcattccaaccttgatgtgttaaactatgtgcaaacaggagggagactggagccaccaagaaattgtcctgatgatctgtggaatttaatgacccagtgctgggctcaagaacccgaccaaagacctacttttcatagaattcaggaccaacttcagttattcagaaattttttcttaaatagcatttataagtccagagatgaagcaaacaacagtggagtcataaatgaaagctttgaaggtgaagatggcgatgtgatttgtttgaattcagatgacattatgccagttgctttaatggaaacgaagaaccgagaagggttaaactatatggtacttgctacagaatgtggccaaggtgaagaaaagtctgagggtcctctaggctcccaggaatctgaatcttgtggtctgaggaaagaagagaaggaaccacatgcagacaaagatttctgccaagaaaaacaagtggcttactgcccttctggcaagcctgaaggcctgaactatgcctgtctcactcacagtggatatggagatgggtctgattaa

SEQ ID NO: 7 - DNA, 2301 bp, Homo sapiens
gtcgaccggagggcaggaggagcaggaggagcaggagcaggaggagcaggaggagcaggaggagcaggaggagcaggaggagcaggaacaggaggaggaggaggaggagaaggaggagcaggaagagcaggaggaggaggagcaggagcaggaggagcaggagggagaggaggctgcaacgccgagcggaggaggcaggaaccggagcgcgagcagtagctgggtgggcaccatggctgggatcaccaccatcgaggcggtgaagcgcaagatccaggttctgcagcagcaggcagatgatgcagaggagcgagctgagcgcctccagcgagaagttgagggagaaaggcgggcccgggaacaggctgaggctgaggtggcctccttgaaccgtaggatccagctggttgaagaagagctggaccgtgctcaggagcgcctggccactgccctgcaaaagctggaagaagctgaaaaagctgctgatgagagtgagagaggtatgaaggttattgaaaaccgggccttaaaagatgaagaaaagatggaactccaggaaatccaactcgaagaagctaagcacattgcagaagaggcagataggaagtatgaagaggtggctcgtaagttggtgatcattgaaggagacttggaacgcacagaggaacgagctgagctggcagagtcgcgttgccgagagatggatgagcagattagactgatggaccagaacctgaagtgtctgagtgctgccgaagaaaagtactctcaaaaagaagataaatatgaggaagaaatcaagattcttactgataaactcaaggaggcagagacccgtgctgagtttgctgagagatcggtagccaagctggaaaagacaattgatgacctggaagacactaacagcacatctggagacccggtggagaagaaggacgaaacaccttttggggtctcggtggctgtgggcctggccgtctttgcctgcctcttcctttctacgctgctccttgtgctcaacaaatgtggacggagaaacaagtttgggatcaaccgcccggctgtgctggctccagaggatgggctggccatgtccctgcatttcatgacattgggtggcagctccctgtcccccaccgagggcaaaggctctgggctccaaggccacatcatcgagaacccacaatacttcagtgatgcctgtgttcaccacatcaagcgccgggacatcgtgctcaagtgggagctgggggagggcgcctttgggaaggtcttccttgctgagtgccacaacctcctgcctgagcaggacaagatgctggtggctgtcaaggcactgaaggaggcgtccgagagtgctcggcaggacttccaacgtgaggctgagctgctcaccatgctgcagcaccagcacatcgtgcgcttcttcggcgtctgcaccgagggccgccccctgctcatggtcttcgagtatatgcggcacggggacctcaaccgcttcctccgatcccatggacccgatgccaagctgctggctggtggggaggatgtggctccaggccccctgggtctggggcagctgctggccgtggctagccaggtcgctgcggggatggtgtacctggcgggtctgcattttgtgcaccgggacctggccacacgcaactgtctagtgggccagggactggtggtcaagattggtgattttggcatgagcagggatatctacagcaccgactattaccgtgtgggaggccgcaccatgctgcccattcgctggatgccgcccgagagcatcctgtaccgtaagttcaccaccgagagcgacgtgtggagcttcggcgtggtgctctgggagatcttcacctacggcaagcagccctggtaccagctctccaacacggaggcaatcgactgcatcacgcagggacgtgagttggagcggccacgtgcctgcccaccagaggtctacgccatcatgcggggctgctggcagcgggagcccagcaacgccacagcatcaaggatgtgcacgcccggctgcaagccctggcctaggcacctcctgtctacctggatgtcctgggctagggggccggcccaggggctgggagtggttagccggaatactggggcctgccctcagcatcccccatagctcccagcagccccagggtgatctcgaagtatctaattcgccctcagcatgtgggaagggacaggtgggggctgggagtagaggatgttcctgcttctctaggcaaggtcccgtcgtagcaattatatttattatgggaattc

SEQ ID NO: 8 - DNA, 2003 bp, Homo sapiens
aacatcctggagtccaccatgaacggacagttggatctaagtgggaagctaatcgtcaaagctcaacttggggaggatattcggcgaattcctattcataatgaagatattacttatgatgaattagtgctaatgatgcaacgagttttcagaggaaaacttctgagtaatgatgaagtaacaataaagtataaagatgaagatggagatcttataacaatttttgatagttctgacctttcctttgcaattcagtgcagtaggatactgaaactgacattatttgttaatggccagccaagaccccttgaatcaagtcaggtgaaatatctccgtcgagaactgatagaacttcgaaataaagtgaatcgtttattggatagcttggaaccacctggagaaccaggaccttccaccaatattcctgaaaatgatactgtggatggtagggaagaaaagtctgcttctgattcttctggaaaacagtctactcaggttatggcagcaagtatgtctgcttttgatcctttaaaaaaccaagatgaaatcaataaaaatgttatgtcagcgtttggcttaacagatgatcaggtttcagacactaacagcacatctggagacccggtggagaagaaggacgaaacaccttttggggtctcggtggctgtgggcctggccgtctttgcctgcctcttcctttctacgctgctccttgtgctcaacaaatgtggacggagaaacaagtttgggatcaaccgcccggctgtcctggctccagaggatgggctggccatgtccctgcatttcatgacattgggtggcagctccctgtcccccaccgagggcaaaggctctgggctccaaggccacatcatcgagaacccacaatacttcagtgatgcctgtgttcaccacatcaagcgccgggacatcgtgctcaagtgggagctgggggagggcgcctttgggaaggtcttccttgctgagtcccacaacctcctgcctgagcaggacaagatgctggtggctgtcaaggcactgaaggaggcgtccgagagtgctcggcaggacttccaacgtgaggctgagctgctcaccatgctgcagcaccagcacatcgtgcgcttcttcggcgtctgcaccgagggccgccccctgctcatggtctttgagtatatgcggcacggggacctcaaccgcttcctccgatcccatggacctgatgccaagctgctggctggtggggaggatgtggctccaggccccctgggtctggggcagctgctggctgtggctagccaggtcgctgcggggatggtgtacctggcgggtctgcattttgtgcaccgggacctggccacacgcaactgtctagtgggccagggactggtggtcaagattggtgattttggcatgagcagggatatctacagcaccgactattaccgtgtgggaggccgcaccatgctgcccattcgctggatgccgcccgagagcatcctgtaccgtaagttcaccaccgagagcgacgtgtggagcttcggcgtggtgctctgggagatcttcacctacggcaagcagccctggtaccagctctccaacacggaggcaatcgactgcatcacgcagggacgtgagttggagcggccacgtgcctgcccaccagaggtctacgccatcatgcggggctgctggcagcgggagccccagcaacgccacagcatcaaggatgtgcacgcccggctgcaagccctggcccaggcacctcctgtctacctggatgtcctgggctagggggccggcccaggggctgggagtggttagccggaatactggggcctgccctcagcatcccccatagctcccagcagccccagggtgatctcgaagtatctaattcgccctcagcatgtgggaagggacaggtgggggctgggagtagaggatgttcctgcttctctaggcaaggtcccgtcatagcaattatatttattatcccttga

SEQ ID NO: 9 - DNA, 2523 bp, Unknown
  Description of Unknown: Genomic polynucleotide
atgcctcacaactccatcagatctggccatggagggctgaaccagctgggaggggcctttgtgaatggcagacctctgccggaagtggtccgccagcgcatcgtagacctggcccaccagggtgtaaggccctgcgacatctctcgccagctccgcgtcagccatggctgcgtcagcaagatccttggcaggtactacgagactggcagcatccggcctggagtgatagggggctccaagcccaaggtggccacccccaaggtggtggagaagattggggactacaaacgccagaaccctaccatgtttgcctgggagatccgagaccggctcctggctgagggcgtctgtgacaatgacactgtgcccagtgtcagctccattaatagaatcatccggaccaaagtgcagcaaccattcaacctccctatggacagctgcgtggccaccaagtccctgagtcccggacacacgctgatccccagctcagctgtaactcccccggagtcaccccagtcggattccctgggctccacctactccatcaatgggctcctgggcatcgctcagcctggcagcgacaagaggaaaatggatgacagtgatcaggatagctgccgactaagcattgactcacagagcagcagcagcggaccccgaaagcaccttcgcacggatgccttcagccagcaccacctcgagccgctcgagtgcccatttgagcggcagcactacccagaggcctatgcctcccccagccacaccaaaggcgagcagggcctctacccgctgcccttgctcaacagcaccctggacgacgggaaggccaccctgaccccttccaacacgccactggggcgcaacctctcgactcaccagacctaccccgtggtggcagatcctcactcacccttggccataaagcaggaaacccccgaggtgtccagttctagctccaccccttgctctttatctagctccgcccttttggatctgcagcaagtcggctccggggtcccgcccttcaatgcctttccccatgctgcctccgtgtacgggcagttcacgggccaggccctcctctcagaaatgaccatggttgacacagagatgccattctggcccaccaactttgggatcagctccgtggatctctccgtaatggaagaccactcccactcctttgatatcaagcccttcactactgttgacttctccagcatttctactccacattacgaagacattccattcacaagaacagatccagtggttgcagattacaagtatgacctgaaacttcaagagtaccaaagtgcaatcaaagtggagcctgcatctccaccttattattctgagaagactcagctctacaataagcctcatgaagagccttccaactccctcatggcaattgaatgtcgtgtctgtggagataaagcttctggatttcactatggagttcatgcttgtgaaggatgcaagggtttcttccggagaacaatcagattgaagcttatctatgacagatgtgatcttaactgtcggatccacaaaaaaagtagaaataaatgtcagtactgtcggtttcagaaatgccttgcagtggggatgtctcataatgccatcaggtttgggcggatgccacaggccgagaaggagaagctgttggcggagatctccagtgatatcgaccagctgaatccagagtccgctgacctccgggccctggcaaaacatttgtatgactcatacataaagtccttcccgctgaccaaagcaaaggcgagggcgatcttgacaggaaagacaacagacaaatcaccattcgttatctatgacatgaattccttaatgatgggagaagataaaatcaagttcaaacacatcacccccctgcaggagcagagcaaagaggtggccatccgcatctttcagggctgccagtttcgctccgtggaggctgtgcaggagatcacagagtatgccaaaagcattcctggttttgtaaatcttgacttgaacgaccaagtaactctcctcaaatatggagtccacgagatcatttacacaatgctggcctccttgatgaataaagatggggttctcatatccgagggccaaggcttcatgacaagggagtttctaaagagcctgcgaaagccttttggtgactttatggagcccaagtttgagtttgctgtgaagttcaatgcactggaattagatgacagcgacttggcaatatttattgctgtcattattctcagtggagaccgcccaggtttgctgaatgtgaagcccattgaagacattcaagacaacctgctacaagccctggagctccagctgaagctgaaccaccctgagtcctcacagctgtttgccaagctgctccagaaaatgacagacctcagacagattgtcacggaacacgtgcagctactgcaggtgatcaagaagacggagacagacatgagtcttcacccgctcctgcaggagatctacaaggacttgtactag

SEQ ID NO: 10 - DNA, 1372 bp, Homo sapiens
gagaacaaccaccaggagtcctaccctctgtcagtgtctcccatggagaataatcactgcccagcgtcctccgagtcccacccgaagccatccagcccccggcaggagagcacacgcgtgatccagctgatgcccagccccatcatgcaccctctgatcctgaacccccggcactccgtggatttcaaacagtccaggctctccgaggacgggctgcatagggaagggaagcccatcaacctctctcatcgggaagacctggcttacatgaaccacatcatggtctctgtctccccgcctgaagagcacgccatgcccattgggagaatagcagatgtgcagcacattaagaggagagacatcgtgctgaagcgagaactgggtgagggagcctttggaaaggtcttcctggccgagtgctacaacctcagcccgaccaaggacaagatgcttgtggctgtgaaggccctgaaggatcccaccctggctgcccggaaggatttccagagggaggccgagctgctcaccaacctgcagcatgagcacattgtcaagttctatggagtgtgcggcgatggggaccccctcatcatggtctttgaatacatgaagcatggagacctgaataagttcctcagggcccatgggccagatgcaatgatccttgtggatggacagccacgccaggccaagggtgagctggggctctcccaaatgctccacattgccagtcagatcgcctcgggtatggtgtacctggcctcccagcactttgtgcaccgagacctggccaccaggaactgcctggttggagcgaatctgctagtgaagattggggacttcggcatgtccagagatgtctacagcacggattattacagggtgggaggacacaccatgctccccattcgctggatgcctcctgaaagcatcatgtaccggaagttcactacagagagtgatgtatggagcttcggggtgatcctctgggagatcttcacctatggaaagcagccatggttccaactctcaaacacggaggtcattgagtgcattacccaaggtcgtgttttggagcggccccgagtctgccccaaagaggtgtacgatgtcatgctggggtgctggcagagggaaccacagcagcggttgaacatcaaggagatctacaaaatcctccatgctttggggaaggccaccccaatctacctggacattcttggctagtggtggctggtggtcatgaattcatactctgttgcctcctctctccctgcctcacatctcccttccacctcacaactccttccatccttgactgaagcgaacatcttcatataaactcaagtgcctgctacacatacaacactga

SEQ ID NO: 11 - DNA, 3237 bp, Artificial Sequence
  Description of Artificial Sequence: Synthetic polynucleotide
atttaggtgacactatagaagtggctgtggagtttcacccaacagatgcaaataccataattacatgcggtaaatctcatattttcttctggacctggagcggcaattcactaacaagaaaacagggaatttttgggaaatatgaaaagccaaaatttgtgcagtgtttagcattcttggggaatggagatgttcttactggagactcaggtggagtcatgcttatatggagcaaaactactgtagagcccacacctgggaaaggacctaaagtgtaccgccggaagcaccaggagctgcaagccatgcagatggagctgcagagccctgagtacaagctgagcaagctccgcacctcgaccatcatgaccgactacaaccccaactactgctttgctggcaagacctcctccatcagtgacctgaaggaggtgccgcggaaaaacatcaccctcattcggggtctgggccatggagcctttggggaggtgtatgaaggccaggtgtccggaatgcccaacgaaatcttgaacagctcactaaagtgcacaaacagttggtacgtgataatgcagatctccgctgtgaacttcctaagttggaaaagcgacttcgagctacagctgagagagtgaaagctttggaatcagcactgaaagaagctaaagaaaatgcatctcgtgatcgcaaacgctatcagcaagaagtagatcgcataaaggaagcagtcaggtcaaagaatatggccagaagagggcattctgcacagattgatccactgtgcgacgagctgtgccgcacggtgatcgcagccgctgtcctcttctccttcatcgtctcggtgctgctgtctgccttctgcatccactgctaccacaagtttgcccacaagccacccatctcctcagctgagatgaccttccggaggcccgcccaggccttcccggtcagctactcctcttccggtgcccgccggccctcgctggactccatggagaaccaggtctccgtggatgccttcaaaggggcccatgcagaatgccaccaagtatggcaacatgacagaggaccatgtgatgcacctgctccagaatgctgaccccctgaaggtgtacccgccactgaaggggagcttcccggagaacctgagacaccttaagaacaccatggagaccatagactggaaggtctttgagagctggatgcaccattggctcctgtttgaaatgagcaggcactccttggagcaaaagcccactgacgctccaccgaaagatgatttttggataccagaaacaagtttcatacttactattatagttggaatatttctggttgttacaatcccactgacctttgtctggcatagaagattaaagaatcaaaaaagtgccaaggaaggggtgacagtgcttataaacgaagacaaagagttggctgagctgcgaggtctggcagccggagtaggcctggctaatgcctgctatgcaatacatactcttccaacccaagaggagattgaaacttggaacgcacagaggaacgagctgagctggcagagtcgcgttgccgagagatggatgagcagattagactgatggaccagaacctgaagtgtctgagtgctgccgaagaaaagtactctcaaaaagaagataaatatgaggaagaaatcaagattcttactgataaactcaaggaggcagagacccgtgctgagtttgctgagagatcggtagccaagctggaaaagacaattgatgacctggaagacactaacagcacatctggagacccggtggagaagaaggacgaaacaccttttggggtctcggtggctgtgggcctggccgtctttgcctgcctcttcctttctacgctgctccttgtgctcaacaaatgtggacggagaaacaagtttgggatcaaccgcccggctgtgctggctccagaggatgggctggccatgtccctgcatttcatgacattgggtggcagctccctgtcccccaccgagggcaaatgacgtctggtcctttggggtcctgctctgggagatcttcacgctggggggctccccgtaccccggcatccctgtggaggagctcttcaagctgctgaaggagggccaccgcatggacaagcccgccaactgcacacacgacctgtacatgatcatgcgggagtgctggcatgccgcgccctcccagaggcccaccttcaagcagctggtggaggacctggaccgtgtccttaccgtgacgtccaccgacaatgttatggaacagttcaatcctgggctgcgaaatttaataaacctggggaaaaattatgagaaagctgtaaacgctatgatcctggcaggaaaagcctactacgatggagtggccaagatcggtgagattgccactgggtcccccgtgtcaactgaactgggacatgtcctcatagagatttcaagtacccacaagaaactcaacgagagtcttgatgaaaattttaaaaaattccacaaagagattaaccccttccaacacgccactggggcgcaacctctcgactcaccagacctaccccgtggtggcagatcctcactcacccttggccataaagcaggaaacccccgaggtgtccagttctagctccaccccttgctctttatctagctccgcccttttggatctgcagcaagtcggctccggggtcccgcccttcaatgcctttccccatgctgcctccgtgtacgggcagttcacgggccaggccctcctctcagaaatgaccatggttgacacagagatgccattctggcccaccaactttgggatcagctccgtggatctctccgtaatggaagaccactcccactcctttgatatcaagcccttcactactgttgacttctccagcatttctactccacattacgaagacattccattcacaagaacagatccagtggttgcagattacaagtatgacctgaaacttcaagagtaccaaagtgcaatcaaagtggagccgaaacaaaggcgtggtttagagtaggtataacaggcactttagcagtggccgtgacgacccggtatgaggtagacaatattacacctgtcctactggcattgagaacttttgcccagagcaaaagtaacttttattatttcttttattaatcaacaaaattttgtttttaacatttcaaaaaaaaaaaaaaaaaaaaaaaaaaaaaaaaaaaaa

SEQ ID NO: 12 - DNA, 3237 bp, Artificial Sequence
  Description of Artificial Sequence: Synthetic polynucleotide
atttaggtgacactatagaagtggatgaaaatgagcaccagttatctttaagaacggtcagtttaggggctggtgcaaaggatgagttgcacattgttgaagcagaggcaatgaattacgaaggcagtccaattaaagtaacactggcaactttgaaaatgtctgtacagccaacggtttcccttgggggctttgaaataacaccaccagtggtcttaaggttgaagtgtggttcagggccagtgcatattagtggacagcacttagtagtgtaccgccggaagcaccaggagctgcaagccatgcagatggagctgcagagccctgagtacaagctgagcaagctccgcacctcgaccatcatgaccgactacaaccccaactactgctttgctggcaagacctcctccatcagtgacctgaaggaggtgccgcggaaaaacatcaccctcattcggggtctgggccatggcgcctttggggaggtgtatgaaggccaggtgtccggaatgcccaacgacccgtctctcaaaaccattcaaattcctgagcacttgatggctcatgctagttcagcaaatattgggcccttcctggagaagagaggctgtatctccatgccagagcagaagtcagcatccggtattgtagctgtccctttcagcgaatggctccttggaagcaaacctgccagtggttatcaagctccttacatacccagcaccgacccccaggactggcttacccaaaagcagaccttggagaacagtcaggaggatccaaagtgggaattccctcggaagaacttggttcttggaaaaactctaggagaaggcgaatttggaaaagtggtcaaggcaacggccttccatctgaaaggcagagcagggtacaccacggtggccgtgaagatgctgaaagagaacgcctccccgagtgagcttcgagacctgctgtcagagttcaacgtcctgaagcaggtcaaccacccacatgtcatcaaattgtatggggcctgcagcctgaggcacctgtaaccaagattgaacttctgccgtcctactccacggctacactgatagatgagcccactgaggtggatgacccctggaacctacccactcttcaggactcggggatcaagtggtcagagagagacaccaaagggaagattctctgtttcttccaagggattgggagattgattttacttctcggatttctctactttttcgtgtgctccctggatattcttagtagcgccttccagctggttggagatgatttttggataccagaaacaagtttcatacttactattatagttggaatatttctggttgttacaatcccactgacctttgtctggcatagaagattaaagaatcaaaaaagtgccaaggaaggggtgacagtgcttataaacgaagacaaagagttggctgagctgcgaggtctggcagccggagtaggcctggctaatgcctgctatgcaatacatactcttccaacccaagaggagaagaacttcgaaataaagtgaatcgtttattggatagcttggaaccacctggagaaccaggaccttccaccaatattcctgaaaatgatactgtggatggtagggaagaaaagtctgcttctgattcttctggaaaacagtctactcaggttatggcagcaagtatgtctgcttttgatcctttaaaaaaccaagatgaaatcaataaaaatgttatgtcagcgtttggcttaacagatgatcaggtttcagacactaacagcacatctggagacccggtggagaagaaggacgaaacaccttttggggtctcggtggctgtgggcctggccgtctttgcctgcctcttcctttctacgctgctccttgtgctcaacaaatgtggacggagaaacaagtttgggatcaaccgcccggctgtcctggctccagaggatgggctggccatgtccctgcatttcatgacattgggtggcagctccctgtcccccaccgagggcatgacgtctggtcctttggggtcctgctctgggagatcttcacgctggggggctccccgtaccccggcatccctgtggaggagctcttcaagctgctgaaggagggccaccgcatggacaagcccgccaactgcacacacgacctgtacatgatcatgcgggagtgctggcatgccgcgccctcccagaggcccaccttcaagcagctggtggaggacctggaccgtgtccttaccgtgacgtccaccgacgtaaaggcgacacaggaggagaaccgggagctgaggagcaggtgtgaggagctccacgggaagaacctggaactggggaagatcatggacaggttcgaagaggttgtgtaccaggccatggaggaagttcagaagcagaaggaactttccaaagctgaaatccagaaagttctaaaagaaaaagaccaacttaccacagatctgaactccatggagaagtccttctccgacctcttcaagcgttttgagaccatccagcccccggcaggagagcacacgcgtgatccagctgatgcccagccccatcatgcaccctctgatcctgaacccccggcactccgtggatttcaaacagtccaggctctccgaggacgggctgcatagggaagggaagcccatcaacctctctcatcgggaagacctggcttacatgaaccacatcatggtctctgtctccccgcctgaagagcacgccatgcccattgggagaatagcagatgtgcagcacattaagaggagagacatcgtgctgaagcgagaactgggtgagggagcctttggaaaggtcttcctggccgagtgctacaacctcagcccgaccaaggacaagatgcttgtggctgtgaaggccctgaaggatcccaccctggctgcccggaaggatttccagagggaggccgagctgctcaccaacctgcagcatgagcacattgtcaagttctatggagtgtgcggcgatggggaccccctgaaacaaaggcgtggtttagagtaggtataacaggcactttagcagtggccgtgacgacccggtatgaggtagacaatattacacctgtcctactggcattgagaacttttgcccagagcaaaagtaacttttattatttcttttattaatcaacaaaattttgtttttaacatttcaaaaaaaaaaaaaaaaaaaaaaaaaaaaaaaaaaaaa

SEQ ID NO: 13 - DNA, 14 bp, Artificial Sequence
  Description of Artificial Sequence: Synthetic oligonucleotide
aaaaaaaaaaaaaa